European Patent Specification EP 3 450 571 B1, published April 5, 2023. Title: METHODS OF USING AN ACTIVATOR OF CEREBLON FOR NEURAL CELL EXPANSION AND THE TREATMENT OF CENTRAL NERVOUS SYSTEM DISORDERS. Applicant: Celgene Corporation. Application TBA. The sequence listing filed with the application follows.

SEQUENCE LISTING (40 sequences)

SEQ ID NO: 1 - DNA, 25 bp, Artificial Sequence
  antagonist of BRD7 - a Morpholino oligonucleotide
tgtgtttcttgtgctttttgcccat

SEQ ID NO: 2 - DNA, 25 bp, Artificial Sequence
  AMO sequence used for the Ikaros gene knockdown
ttcctgtgcctcctcagtctccatc

SEQ ID NO: 3 - DNA, 25 bp, Artificial Sequence
  AMO sequence used for the CRBN gene knockdown
agagctgtagctggttccccatttc

SEQ ID NO: 4 - DNA, 25 bp, Artificial Sequence
  AMO sequence used for the Lhx2 gene knockdown
tctgcaacccaagatttccgtgaga

SEQ ID NO: 5 - DNA, 29 bp, Artificial Sequence
  forward primer for cloning BRD7 gene into pCS2+ vector
tttaagcttatgggcaaaaagcacaagaa

SEQ ID NO: 6 - DNA, 30 bp, Artificial Sequence
  reverse primer for cloning BRD7 gene into pCS2+ vector
ttttctagatcagctcctacgacgcgtgca

SEQ ID NO: 7 - DNA, 34 bp, Artificial Sequence
  forward primer for cloning Ikaros gene into pCS2+ vector
tttgaattcatggagactgaggaggcacaggaaa

SEQ ID NO: 8 - DNA, 33 bp, Artificial Sequence
  reverse primer for cloning Ikaros gene into pCS2+ vector
tttctcgagtcagatgcggtgctctccacgtgt

SEQ ID NO: 9 - DNA, 21 bp, Artificial Sequence
  forward primer used in reverse transcription of Quantitative PCR
aaggctatcaacacgctcaac

SEQ ID NO: 10 - DNA, 20 bp, Artificial Sequence
  reverse primer used in reverse transcription of Quantitative PCR
tcacatacaggttggcatcg

SEQ ID NO: 11 - DNA, 1488 bp, Artificial Sequence
  nucleotide sequence of ikzf1-006 Ikaros variant
  misc_feature 808: n = A,T,C or G
atggagactgaggaggcacaggaaatgtcccagataacaggaagagacagcccgatgaatgctaatgaaggcggagaggatcaagatgaggccatgcctgttcctgaagacttgtcagcaagcactggcctccaacacaacaatcgcacagataaaccactggcctgtaatataaaagttgaggctcggagtgacgaggaaaacggtctgtcctgtgagatgaatggagaggcagaggaatgtgcagctgaggacttgcgcatactcgatggctctggggccaaagtgaacggctcccacgcaggccccgacagcaagccggccgcctaccccacagccgggggcatccgcctccccaacgggaagctgaagtgcgatatctgtgggatagtttgcattgggcccaatgtgttgatggttcacaagcgaagtcacactgaagaaagaaagtcagttttggaacaacaaaaaggtgaaaggccattccagtgcaatcaatgtggtgcttcattcactcagaagggtaacctgctccgacacatcaaacttcactctggcgagaaacctttcaaatgtcacctgtgcaactatgcttgccgccgcagagacgctctcactggacatctgcgcactcattcggttggaaagccccataagtgtgcatattgcggacgcagttacaagcagcggagctcactggaggaacataaggagagatgtcacaactacttgcagtgcatgggccttcagaacagcatttatacaggagagaatcgtctgtcagagctatctttcgagagtggctcangtgagctgatgcagccccatgtgattgatcaggccatcaacagtgcaattagctatctgggtgcagagtccttgcggcctctggttcagacctctcctgggtccgccgacatggtggtcagccctctatacaacctgcacaagtcacaaacagctgaaggcaatggtgtttctgctaaagacagcgccgcagagcaccttctcctactctctaagtccaaatccgcctctgttgacaaagacggttcccccagtcccagcgggcaggattccactgacactgagagcaacaacgaggagcgttcggccggggtaagcggaacagcagccacaggtggtctcatctacctgaccaaccacatggctccaggtatgagaaatggaggcctgccaggggtaaaggaagaacaacaccggcagtttgaggctttgcgagcagcaggaatggatttgagtatagcgtcatcagaaggatttaaggtgctaagtggagatggagaagaattgagggcgtaccgctgtatccactgcagagttttgttcctggatcatgtcatgtacaccatccacatgggctgtcatggcttccgagacccctttgagtgcaacctatgcgggtaccgcagtcaggaccgttatgagttctcatcgcacatcacacgtggagagcaccgcatctga

SEQ ID NO: 12 - protein, 495 aa, Artificial Sequence
  amino acid sequence of ikzf1-006 Ikaros variant
  VARIANT 270: Xaa = Any Amino Acid
METEEAQEMSQITGRDSPMNANEGGEDQDEAMPVPEDLSASTGLQHNNRTDKPLACNIKVEARSDEENGLSCEMNGEAEECAAEDLRILDGSGAKVNGSHAGPDSKPAAYPTAGGIRLPNGKLKCDICGIVCIGPNVLMVHKRSHTEERKSVLEQQKGERPFQCNQCGASFTQKGNLLRHIKLHSGEKPFKCHLCNYACRRRDALTGHLRTHSVGKPHKCAYCGRSYKQRSSLEEHKERCHNYLQCMGLQNSIYTGENRLSELSFESGSXELMQPHVIDQAINSAISYLGAESLRPLVQTSPGSADMVVSPLYNLHKSQTAEGNGVSAKDSAAEHLLLLSKSKSASVDKDGSPSPSGQDSTDTESNNEERSAGVSGTAATGGLIYLTNHMAPGMRNGGLPGVKEEQHRQFEALRAAGMDLSIASSEGFKVLSGDGEELRAYRCIHCRVLFLDHVMYTIHMGCHGFRDPFECNLCGYRSQDRYEFSSHITRGEHRI

SEQ ID NO: 13 - DNA, 1455 bp, Artificial Sequence
  nucleotide sequence of ikzf1-007 Ikaros variant
  misc_feature 775: n = A,T,C or G
atggagactgaggaggcacaggaaatgtcccagataacaggaagagacagcccgatgaatgctaatgaaggcggagaggatcaagatgaggccatgcctgttcctgaagacttgtcagcaagcactggcctccaacacaacaatcgcacagataaaccactggcctgtaatataaaagttgaggctcggagtgacgaggaaaacggtctgtcctgtgagatgaatggagaggcagaggaatgtgcagctgaggacttgcgcatactcgatggctctggggccaaagtgaacggctcccacgcaggccccgacagcaagccggccgcctaccccacagccgggggcatccgcctccccaacgggaagctgaagtgcgatatctgtgggatagtttgcattgggcccaatgtgttgatggttcacaagcgaagtcacactggtgaaaggccattccagtgcaatcaatgtggtgcttcattcactcagaagggtaacctgctccgacacatcaaacttcactctggcgagaaacctttcaaatgtcacctgtgcaactatgcttgccgccgcagagacgctctcactggacatctgcgcactcattcggttggaaagccccataagtgtgcatattgcggacgcagttacaagcagcggagctcactggaggaacataaggagagatgtcacaactacttgcagtgcatgggccttcagaacagcatttatacaggagagaatcgtctgtcagagctatctttcgagagtggctcangtgagctgatgcagccccatgtgattgatcaggccatcaacagtgcaattagctatctgggtgcagagtccttgcggcctctggttcagacctctcctgggtccgccgacatggtggtcagccctctatacaacctgcacaagtcacaaacagctgaaggcaatggtgtttctgctaaagacagcgccgcagagcaccttctcctactctctaagtccaaatccgcctctgttgacaaagacggttcccccagtcccagcgggcaggattccactgacactgagagcaacaacgaggagcgttcggccggggtaagcggaacagcagccacaggtggtctcatctacctgaccaaccacatggctccaggtatgagaaatggaggcctgccaggggtaaaggaagaacaacaccggcagtttgaggctttgcgagcagcaggaatggatttgagtatagcgtcatcagaaggatttaaggtgctaagtggagatggagaagaattgagggcgtaccgctgtatccactgcagagttttgttcctggatcatgtcatgtacaccatccacatgggctgtcatggcttccgagacccctttgagtgcaacctatgcgggtaccgcagtcaggaccgttatgagttctcatcgcacatcacacgtggagagcaccgcatctga

SEQ ID NO: 14 - protein, 484 aa, Artificial Sequence
  amino acid sequence of ikzf1-007 Ikaros variant
  VARIANT 259: Xaa = Any Amino Acid
METEEAQEMSQITGRDSPMNANEGGEDQDEAMPVPEDLSASTGLQHNNRTDKPLACNIKVEARSDEENGLSCEMNGEAEECAAEDLRILDGSGAKVNGSHAGPDSKPAAYPTAGGIRLPNGKLKCDICGIVCIGPNVLMVHKRSHTGERPFQCNQCGASFTQKGNLLRHIKLHSGEKPFKCHLCNYACRRRDALTGHLRTHSVGKPHKCAYCGRSYKQRSSLEEHKERCHNYLQCMGLQNSIYTGENRLSELSFESGSXELMQPHVIDQAINSAISYLGAESLRPLVQTSPGSADMVVSPLYNLHKSQTAEGNGVSAKDSAAEHLLLLSKSKSASVDKDGSPSPSGQDSTDTESNNEERSAGVSGTAATGGLIYLTNHMAPGMRNGGLPGVKEEQHRQFEALRAAGMDLSIASSEGFKVLSGDGEELRAYRCIHCRVLFLDHVMYTIHMGCHGFRDPFECNLCGYRSQDRYEFSSHITRGEHRI

SEQ ID NO: 15 - DNA, 21 bp, Artificial Sequence
  forward primer of quantitative PCR of c-Myc
aacagctatgaccatgattac

SEQ ID NO: 16 - DNA, 17 bp, Artificial Sequence
  reverse primer of quantitative PCR of c-Myc
gtaaaacgacggccagt

SEQ ID NO: 17 - DNA, 18 bp, Artificial Sequence
  forward primer of quantitative PCR of sox2
accccggaggaaaaccaa

SEQ ID NO: 18 - DNA, 18 bp, Artificial Sequence
  reverse primer of quantitative PCR of sox2
cccggcagggtgtacttg

SEQ ID NO: 19 - DNA, 19 bp, Artificial Sequence
  forward primer of quantitative PCR of nanog
tacccaacacaccagcttc

SEQ ID NO: 20 - DNA, 19 bp, Artificial Sequence
  reverse primer of quantitative PCR of nanog
gaagggtgtttttggagga

SEQ ID NO: 21 - DNA, 17 bp, Artificial Sequence
  forward primer for amplification of Ascl1a
acgagcatgacgccgta

SEQ ID NO: 22 - DNA, 25 bp, Artificial Sequence
  reverse primer for amplification of Ascl1a
ttttaagtttccttttacgaacgct

SEQ ID NO: 23 - DNA, 20 bp, Artificial Sequence
  forward primer for amplification of Pou3f2b
ccgagagtcatggcgactac

SEQ ID NO: 24 - DNA, 20 bp, Artificial Sequence
  reverse primer for amplification of Pou3f2b
cttctccgtgtgacaaggct

SEQ ID NO: 25 - DNA, 20 bp, Artificial Sequence
  forward primer for amplification of Myt1la
actcaacagccactgctacc

SEQ ID NO: 26 - DNA, 20 bp, Artificial Sequence
  reverse primer for amplification of Myt1la
agcttgatagcgtgaggagc

SEQ ID NO: 27 - DNA, 20 bp, Artificial Sequence
  forward primer for amplification of Notch3
acaacagcgaaggattgctc

SEQ ID NO: 28 - DNA, 20 bp, Artificial Sequence
  reverse primer for amplification of Notch3
tctaaagcctcgctgacaca

SEQ ID NO: 29 - DNA, 20 bp, Artificial Sequence
  forward primer for amplification of Nrp2b
ccagcggatcgtcttaaact

SEQ ID NO: 30 - DNA, 20 bp, Artificial Sequence
  reverse primer for amplification of Nrp2b
caaaactgggcctgaggata

SEQ ID NO: 31 - DNA, 20 bp, Artificial Sequence
  forward primer used in quantitative PCR for Pou5f1
aactgaagccgttgttgcag

SEQ ID NO: 32 - DNA, 20 bp, Artificial Sequence
  reverse primer used in quantitative PCR for Pou5f1
caagctggtccttcgttttc

SEQ ID NO: 33 - DNA, 17 bp, Artificial Sequence
  forward primer used in quantitative PCR for Zic3
ccctgggctgggactca

SEQ ID NO: 34 - DNA, 19 bp, Artificial Sequence
  reverse primer used in quantitative PCR for Zic3
cttgaaggcagccgagtga

SEQ ID NO: 35 - DNA, 20 bp, Artificial Sequence
  forward primer used in quantitative PCR for CRBN
agaggtcagcatgtttcgca

SEQ ID NO: 36 - DNA, 20 bp, Artificial Sequence
  reverse primer used in quantitative PCR for CRBN
ctgacgaatcccgtctgctt

SEQ ID NO: 37 - DNA, 20 bp, Artificial Sequence
  forward primer used in quantitative PCR for Wnt3a
gcttctgccgcaactatgtg

SEQ ID NO: 38 - DNA, 20 bp, Artificial Sequence
  reverse primer used in quantitative PCR for Wnt3a
ccgattctctggtggccttt

SEQ ID NO: 39 - DNA, 20 bp, Artificial Sequence
  forward primer used in quantitative PCR for Lhx2b
gggggaaacagagacgaaca

SEQ ID NO: 40 - DNA, 21 bp, Artificial Sequence
  reverse primer used in quantitative PCR for Lhx2b
tctctgcaccgaaaaccttct